European Patent Application EP 4 501 954 A1, published February 5, 2025. Title: A nucleic acid encoding a CD8 alpha beta co-receptor, cells and pharmaceutical compositions comprising the same. Applicant: Max-Delbrueck-Centrum fuer Molekulare Medizin in der Helmholtz-Gemeinschaft. The sequence listing filed with the application follows.

SEQUENCE LISTING (24 sequences)

SEQ ID NO: 1 - protein, 243 aa, Homo sapiens
  source 1..243: note = amino acid sequence of human CD8 beta chain isoform 5
MRPRLWLLLAAQLTVLHGNSVLQQTPAYIKVQTNKMVMLSCEAKISLSNMRIYWLRQRQAPSSDSHHEFLALWDSAKGTIHGEEVEQEKIAVFRDASRFILNLTSVKPEDSGIYFCMIVGSPELTFGKGTQLSVVDFLPTTAQPTKKSTLKKRVCRLPRPETQKGPLCSPITLGLLVAGVLVLLVSLGVAIHLCCRRRRARLRFMKQPQGEGISGTFVPQCLHGYYSNTTTSQKLLNPWILKT

SEQ ID NO: 2 - protein, 235 aa, Homo sapiens
  source 1..235: note = amino acid sequence of human CD8 alpha chain isoform 1
MALPVTALLLPLALLLHAARPSQFRVSPLDRTWNLGETVELKCQVLLSNPTSGCSWLFQPRGAAASPTFLLYLSQNKPKAAEGLDTQRFSGKRLGDTFVLTLSDFRRENEGYYFCSALSNSIMYFSHFVPVFLPAKPTTTPAPRPPTPAPTIASQPLSLRPEACRPAAGGAVHTRGLDFACDIYIWAPLAGTCGVLLLSLVITLYCNHRNRRRVCKCPRPVVKSGDKPSLSARYV

SEQ ID NO: 3 - protein, 18 aa, Thosea asigna virus
  source 1..18: note = T2A
EGRGSLLTCGDVEENPGP

SEQ ID NO: 4 - protein, 19 aa, Teschovirus A
  source 1..19: note = P2A
ATNFSLLKQAGDVEENPGP

SEQ ID NO: 5 - protein, 20 aa, Equine rhinitis A virus
  source 1..20: note = E2A
QCTNYALLKLAGDVESNPGP

SEQ ID NO: 6 - protein, 22 aa, Foot-and-mouth disease virus
  source 1..22: note = F2A
VKQTLNFDLLKLAGDVESNPGP

SEQ ID NO: 7 - protein, 8 aa, synthetic construct
  source 1..8: note = core sequence motif of 2A elements peptides
DXEXNPGP

SEQ ID NO: 8 - protein, 7 aa, synthetic construct
  source 1..7: note = consensus TEV cleavage site
ENLYFQS

SEQ ID NO: 9 - DNA, 575 bp, synthetic construct
  source 1..575: mol_type = other DNA; note = preferred IRES
cccccccccctaacgttactggccgaagccgcttggaataaggccggtgtgcgtttgtctatatgttattttccaccatattgccgtcttttggcaatgtgagggcccggaaacctggccctgtcttcttgacgagcattcctaggggtctttcccctctcgccaaaggaatgcaaggtctgttgaatgtcgtgaaggaagcagttcctctggaagcttcttgaagacaaacaacgtctgtagcgaccctttgcaggcagcggaaccccccacctggcgacaggtgcctctgcggccaaaagccacgtgtataagatacacctgcaaaggcggcacaaccccagtgccacgttgtgagttggatagttgtggaaagagtcaaatggctctcctcaagcgtattcaacaaggggctgaaggatgcccagaaggtaccccattgtatgggatctgatctggggcctcggtgcacatgctttacatgtgtttagtcgaggttaaaaaacgtctaggccccccgaaccacggggacgtggttttcctttgaaaaacacgatgataatatggccacaacc

SEQ ID NO: 10 - DNA, 1503 bp, synthetic construct
  source 1..1503: mol_type = other DNA; note = nucleic acid segments encoding the CD8 beta chain linked, via a nucleic acid segment encoding a P2A cleavage site , to the nucleic acid segment encoding the CD8 alpha chain, codon-optimized
atgcggcccagactgtggctgcttcttgctgcacagctgacagtcctgcacggcaatagcgtgctgcaacagaccccagcctacatcaaggtgcagaccaacaagatggtcatgctgagctgcgaggccaagatcagcctgtccaacatgagaatctactggctgcggcagaggcaggccccttcttctgattcccaccacgagtttctggccctgtgggattctgccaagggcacaattcacggcgaggaagtggaacaagagaaaatcgccgtgttccgggacgccagccggttcatcctgaatctgacaagcgtgaagcccgaggacagcggaatctacttctgcatgatcgtgggcagcccagagctgaccttcggaaagggaactcagctgtctgtggtggacttcctgcctaccaccgctcagcccaccaaaaagagcaccctgaagaaacgcgtgtgcagactgcccagaccagagacacagaaaggccctctgtgcagccctatcacactgggattgctggttgccggcgttctggtgctgcttgtgtcactgggagttgccatccacctgtgctgcagacgcagacgggctagactgcggttcatgaagcagcctcaaggcgagggcatctccggcacatttgtgcctcaatgtctgcacggctactacagcaacaccaccaccagccagaagctgctgaacccctggatcctgaaaaccggctccggggccacaaactttagtctgctgaagcaagctggcgacgttgaagaaaatcctgggccaatggcactgcccgtgacagctctgctgcttcctcttgcactgctgctgcatgccgccagacctagccagtttagagtgtcccctctggacagaacctggaacctgggagagacagtggaactgaagtgccaggtcctgctgagcaatcctaccagcggctgcagctggctgtttcagccaagaggtgctgccgcctctcctacctttctgctgtacctgagccagaacaagcccaaggccgccgaaggactggacacccagagattcagcggaaagagactgggcgataccttcgtgctgaccctgtccgacttcagaagagagaacgagggctactacttctgtagcgccctgagcaacagcatcatgtacttctcccacttcgtgcccgtgtttctgcccgccaagcctacaacaacccctgctcctagacctcctacaccagctcctacaatcgccagccagcctctgtctctgaggcctgaagcttgtagacctgctgcaggcggagccgtgcatacaagaggactggatttcgcctgcgacatctacatctgggcccctctggctggaacatgcggagttctgctgctgtccctcgtgatcaccctgtactgcaaccaccggaacaggcggagagtgtgcaagtgccctagacctgtggtcaagagcggcgacaagccttctctgagcgccagatatgtttga

SEQ ID NO: 11 - DNA, 3369 bp, synthetic construct
  source 1..3369: mol_type = other DNA; note = nucleic acid of the invention (operon with CTC127 in the configuration TCRbeta-P2A-TCRalpha-P2A-CD8beta-P2A-CD8alpha)
atgggatctagactgctttgttgggtgctgctgtgcctgcttggagccggacctgtgaaagctggcgtgacccagacacctagatacctgatcaagaccagaggccagcaagtgaccctgagctgctctcctatcagcggccacagaagcgtgtcctggtatcagcagacacctggacagggcctgcagttcctgttcgagtacttcagcgagacacagcggaacaagggcaacttccccggcagattttccggcagacagttcagcaacagccgcagcgagatgaacgtgtccacactggaactgggcgacagcgccctgtatctgtgtgcctcttctcttgccggaactggcgcccacttcatcaccaacgagaagctgttcttcggcagcggcacacagctgagcgtgctggaagatctgagaaacgtgacccctcctaaggtgtccctgtttgagcctagcaaggccgagatcgccaacaagcagaaagccacactcgtgtgcctggccagaggcttctttcccgatcacgtggaactgtcttggtgggtcaacggcaaagaggtgcacagcggcgtctgtacagatccccaggcctacaaagagagcaactacagctactgcctgagcagcagactgagagtgtccgccaccttctggcacaaccccagaaaccacttcagatgccaggtgcagtttcacggcctgagcgaagaggacaagtggcctgagggctctcccaagcctgtgacacagaatatctctgccgaagcctggggcagagccgattgtggaattaccagcgccagctaccatcagggcgtgctgtctgccacaatcctgtacgagatcctgctgggcaaagccactctgtacgccgtgctggtgtctggcctggtgctgatggccatggtcaagaagaagaactctggcagcggcgccaccaacttcagcctgcttaaacaggcaggcgacgtggaagagaaccccggacctatgctgctggaacacctcctgatcatcctgtggatgcagctgacatgggtgtccggccagcagctgaatcagagcccacagagcatgttcatccaagaaggcgaggacgtttccatgaactgcaccagcagcagcatcttcaacacctggctgtggtacaagcaagagcctggcgaaggacccgtgctgctgattgccttgtataaggccggcgagctgaccagcaacggcagactgacagcccagttcggcattacccggaaggacagcttcctgaacatctccgccagcattcccagcgacgtgggcatctatttttgtgccggacagctgtggggcggctccaactacaagctgacatttggcaagggcaccctgctgaccgtgaatcccaacattcagaaccccgagcctgccgtgtaccagctgaaggatcctagaagccaggacagcaccctgtgcctgttcaccgacttcgacagccagatcaacgtgcccaagaccatggaaagcggcacctttatcaccgacaagtgcgtgctggacatgaaggccatggacagcaagagcaacggcgccattgcctggtccaaccagaccagcttcacgtgccaggacatcttcaaagagacaaacgccacctatcctagctccgacgtgccctgtgatgccacactgaccgagaagtccttcgagacagacatgaacctgaacttccagaacctgagcgtgatgggcctgagaatcctgctgctgaaggtggccggcttcaacctgctgatgacactgagactgtggtccagcggatctggagcaacaaacttctcactactcaaacaagcaggtgacgtggaggagaatcccgggcctatgcggccacggctgtggctcctcctggccgcgcagctgacagttctccatggcaactcagtcctccagcagacccctgcatacataaaggtgcaaaccaacaagatggtgatgctgtcctgcgaggctaaaatctccctcagtaacatgcgcatctactggctgagacagcgccaggcaccgagcagtgacagtcaccacgagttcctggccctctgggattccgcaaaagggactatccacggtgaagaggtggaacaggagaagatagctgtgtttcgggatgcaagccggttcattctcaatctcacaagcgtgaagccggaagacagtggcatctacttctgcatgatcgtcgggagccccgagctgaccttcgggaagggaactcagctgagtgtggttgatttccttcccaccactgcccagcccaccaagaagtccaccctcaagaagagagtgtgccggttacccaggccagagacccagaagggcccactttgtagccccatcacccttggcctgctggtggctggcgtcctggttctgctggtttccctgggagtggccatccacctgtgctgccggcggaggagagcccggcttcgtttcatgaaacagcctcaaggggaaggtatatcaggaacctttgtcccccaatgcctgcatggatactacagcaatactacaacctcacagaagctgcttaacccatggatcctgaaaacaggaagcggcgccacaaatttcagcctgctgaaacaggccggcgacgtggaagagaaccctggacctatggccttaccagtgaccgccttgctcctgccgctggccttgctgctccacgccgccaggccgagccagttccgggtgtcgccgctggatcggacctggaacctgggcgagacagtggagctgaagtgccaggtgctgctgtccaacccgacgtcgggctgctcgtggctcttccagccgcgcggcgccgccgccagtcccaccttcctcctatacctctcccaaaacaagcccaaggcggccgaggggctggacacccagcggttctcgggcaagaggttgggggacaccttcgtcctcaccctgagcgacttccgccgagagaacgagggctattatttctgctcggccctgagcaactccatcatgtacttcagccacttcgtgccggtcttcctgccagcgaagcccaccacgacgccagcgccgcgaccaccaacaccggcgcccaccatcgcgtcgcagcccctgtccctgcgcccagaggcgtgccggccagcggcggggggcgcagtgcacacgagggggctggacttcgcctgtgatatctacatctgggcgcccttggccgggacttgtggagtccttctcctgtcactggttatcaccctttactgcaaccacaggaaccgaagacgtgtttgcaaatgtccccggcctgtggtcaaatcgggagacaagcccagcctttcggcgagatacgtc

SEQ ID NO: 12 - DNA, 3372 bp, synthetic construct
  source 1..3372: mol_type = other DNA; note = comparative nucleic acid in the configuration TCRbeta-P2A-TCRalpha-P2A-CD8alpha-P2A-CD8beta (TCR127)
atgggatctagactgctttgttgggtgctgctgtgcctgcttggagccggacctgtgaaagctggcgtgacccagacacctagatacctgatcaagaccagaggccagcaagtgaccctgagctgctctcctatcagcggccacagaagcgtgtcctggtatcagcagacacctggacagggcctgcagttcctgttcgagtacttcagcgagacacagcggaacaagggcaacttccccggcagattttccggcagacagttcagcaacagccgcagcgagatgaacgtgtccacactggaactgggcgacagcgccctgtatctgtgtgcctcttctcttgccggaactggcgcccacttcatcaccaacgagaagctgttcttcggcagcggcacacagctgagcgtgctggaagatctgagaaacgtgacccctcctaaggtgtccctgtttgagcctagcaaggccgagatcgccaacaagcagaaagccacactcgtgtgcctggccagaggcttctttcccgatcacgtggaactgtcttggtgggtcaacggcaaagaggtgcacagcggcgtctgtactgatccccaggcctacaaagagagcaactacagctactgcctgagcagcagactgagagtgtccgccaccttctggcacaaccccagaaaccacttcagatgccaggtgcagtttcacggcctgagcgaagaggacaagtggcctgagggaagccccaagcctgtgacacagaatatctctgccgaagcctggggcagagccgattgtggaattaccagcgccagctaccatcagggcgtgctgtctgccacaatcctgtacgagatcctgctgggcaaagccactctgtacgccgtgctggtgtctggcctggtgctgatggccatggtcaagaagaagaactctggcagcggcgccaccaacttcagcctgcttaaacaggcaggcgacgtggaagagaaccccggacctatgctgctggaacacctcctgatcatcctgtggatgcagctgacatgggtgtccggccagcagctgaatcagagccctcagagcatgttcatccaagaaggcgaggacgtttccatgaactgcaccagcagcagcatcttcaacacctggctgtggtacaagcaagagcctggcgaaggacccgtgctgctgattgccttgtataaggccggcgagctgaccagcaacggcagactgacagcccagttcggcattacccggaaggacagcttcctgaacatctccgccagcattcccagcgacgtgggcatctatttttgtgccggacagctgtggggcggctccaactacaagctgacatttggcaagggcaccctgctgaccgtgaatcccaacattcagaaccccgagcctgccgtgtaccagctgaaggatcctagaagccaggacagcaccctgtgcctgttcaccgacttcgacagccagatcaacgtgcccaagaccatggaaagcggcacctttatcaccgataagtgtgtgctggacatgaaggccatggacagcaagagcaacggcgccattgcctggtccaaccagaccagcttcacgtgccaggacatcttcaaagagacaaacgccacctatcctagctccgacgtgccctgtgatgccacactgaccgagaagtccttcgagacagacatgaacctgaacttccagaacctgagcgtgatgggcctgagaatcctgctgctgaaggtggccggcttcaacctgctgatgacactgagactgtggtcctctggctctggcgctacaaatttctcactgctcaagcaggccggggatgtcgaagagaatccaggaccaatggcactgcccgtgacagctctgctgcttcctcttgcactgctgctgcatgccgccagacctagccagtttagagtgtcccctctggacagaacctggaacctgggagagacagtggaactgaagtgccaggtcctgctgagcaatcctaccagcggctgcagctggctgtttcagccaagaggtgctgccgcctctcctacctttctgctgtacctgagccagaacaagcccaaggccgccgaaggactggacacccagagattcagcggaaagagactgggcgataccttcgtgctgaccctgtccgacttcagaagagagaacgagggctactacttctgtagcgccctgagcaacagcatcatgtacttctcccacttcgtgcccgtgtttctgcccgccaagcctacaacaacccctgctcctagacctcctacaccagctcctacaatcgccagccagcctctgtctctgaggcctgaagcttgtagacctgctgcaggcggagccgtgcatacaagaggactggatttcgcctgcgacatctacatctgggcccctctggctggaacatgcggagttctgctgctgtccctcgtgatcaccctgtactgcaaccaccggaacaggcggagagtgtgcaagtgccctagacctgtggtcaagagcggcgacaagccttctctgagcgccagatatgttggctccggggccacaaactttagtctgctgaagcaagctggcgacgttgaagaaaatcctgggccaatgcggcccagactgtggctgcttcttgctgcacagctgacagtcctgcacggcaatagcgtgctgcaacagaccccagcctacatcaaggtgcagaccaacaagatggtcatgctgagctgcgaggccaagatcagcctgtccaacatgagaatctactggctgcggcagaggcaggccccttcttctgattcccaccacgagtttctggccctgtgggattctgccaagggcacaattcacggcgaggaagtggaacaagagaaaatcgccgtgttccgggacgccagccggttcatcctgaatctgacaagcgtgaagcccgaggacagcggaatctacttctgcatgatcgtgggcagcccagagctgaccttcggaaagggaactcagctgtctgtggtggacttcctgcctaccaccgctcagcccaccaaaaagagcaccctgaagaaacgcgtgtgcagactgcccagaccagagacacagaaaggccctctgtgcagccctatcacactgggattgctggttgccggcgttctggtgctgcttgtgtcactgggagttgccatccacctgtgctgcagacgcagacgggctagactgcggttcatgaagcagcctcaaggcgagggcatctccggcacatttgtgcctcaatgtctgcacggctactacagcaacaccaccaccagccagaagctgctgaacccctggatcctgaaaacctga

SEQ ID NO: 13 - DNA, 2577 bp, synthetic construct
  source 1..2577: mol_type = other DNA; note = comparative nucleic acid in the configuration TCRbeta-P2A-TCRalpha-P2A-CD8alpha (TCR127)
atgggatctagactgctttgttgggtgctgctgtgcctgcttggagccggacctgtgaaagctggcgtgacccagacacctagatacctgatcaagaccagaggccagcaagtgaccctgagctgctctcctatcagcggccacagaagcgtgtcctggtatcagcagacacctggacagggcctgcagttcctgttcgagtacttcagcgagacacagcggaacaagggcaacttccccggcagattttccggcagacagttcagcaacagccgcagcgagatgaacgtgtccacactggaactgggcgacagcgccctgtatctgtgtgcctcttctcttgccggaactggcgcccacttcatcaccaacgagaagctgttcttcggcagcggcacacagctgagcgtgctggaagatctgagaaacgtgacccctcctaaggtgtccctgtttgagcctagcaaggccgagatcgccaacaagcagaaagccacactcgtgtgcctggccagaggcttctttcccgatcacgtggaactgtcttggtgggtcaacggcaaagaggtgcacagcggcgtctgtacagatccccaggcctacaaagagagcaactacagctactgcctgagcagcagactgagagtgtccgccaccttctggcacaaccccagaaaccacttcagatgccaggtgcagtttcacggcctgagcgaagaggacaagtggcctgagggctctcccaagcctgtgacacagaatatctctgccgaagcctggggcagagccgattgtggaattaccagcgccagctaccatcagggcgtgctgtctgccacaatcctgtacgagatcctgctgggcaaagccactctgtacgccgtgctggtgtctggcctggtgctgatggccatggtcaagaagaagaactctggcagcggcgccaccaacttcagcctgcttaaacaggcaggcgacgtggaagagaaccccggacctatgctgctggaacacctcctgatcatcctgtggatgcagctgacatgggtgtccggccagcagctgaatcagagcccacagagcatgttcatccaagaaggcgaggacgtttccatgaactgcaccagcagcagcatcttcaacacctggctgtggtacaagcaagagcctggcgaaggacccgtgctgctgattgccttgtataaggccggcgagctgaccagcaacggcagactgacagcccagttcggcattacccggaaggacagcttcctgaacatctccgccagcattcccagcgacgtgggcatctatttttgtgccggacagctgtggggcggctccaactacaagctgacatttggcaagggcaccctgctgaccgtgaatcccaacattcagaaccccgagcctgccgtgtaccagctgaaggatcctagaagccaggacagcaccctgtgcctgttcaccgacttcgacagccagatcaacgtgcccaagaccatggaaagcggcacctttatcaccgacaagtgcgtgctggacatgaaggccatggacagcaagagcaacggcgccattgcctggtccaaccagaccagcttcacgtgccaggacatcttcaaagagacaaacgccacctatcctagctccgacgtgccctgtgatgccacactgaccgagaagtccttcgagacagacatgaacctgaacttccagaacctgagcgtgatgggcctgagaatcctgctgctgaaggtggccggcttcaacctgctgatgacactgagactgtggtccagcggaagcggcgccacaaatttcagcctgctgaaacaggccggcgacgtggaagagaaccctggacctatggccttaccagtgaccgccttgctcctgccgctggccttgctgctccacgccgccaggccgagccagttccgggtgtcgccgctggatcggacctggaacctgggcgagacagtggagctgaagtgccaggtgctgctgtccaacccgacgtcgggctgctcgtggctcttccagccgcgcggcgccgccgccagtcccaccttcctcctatacctctcccaaaacaagcccaaggcggccgaggggctggacacccagcggttctcgggcaagaggttgggggacaccttcgtcctcaccctgagcgacttccgccgagagaacgagggctattatttctgctcggccctgagcaactccatcatgtacttcagccacttcgtgccggtcttcctgccagcgaagcccaccacgacgccagcgccgcgaccaccaacaccggcgcccaccatcgcgtcgcagcccctgtccctgcgcccagaggcgtgccggccagcggcggggggcgcagtgcacacgagggggctggacttcgcctgtgatatctacatctgggcgcccttggccgggacttgtggagtccttctcctgtcactggttatcaccctttactgcaaccacaggaaccgaagacgtgtttgcaaatgtccccggcctgtggtcaaatcgggagacaagcccagcctttcggcgagatacgtctag

SEQ ID NO: 14 - DNA, 3369 bp, synthetic construct
  source 1..3369: mol_type = other DNA; note = nucleic acid in the configuration CD8beta-P2A-CD8alpha-P2A- TCRbeta-P2A-TCRalpha (TCR127)
atgaggcctagactttggttgctgctggccgctcagctgacagtgctgcacggaaattctgtcctgcagcagacccctgcctacatcaaggtgcagaccaacaagatggtcatgctgagctgcgaggccaagatcagcctgagcaacatgcggatctactggctgcggcagagacaggcccctagctctgatagccaccacgagtttctggccctgtgggattctgccaagggcaccattcacggcgaggaagtggaacaagagaagatcgccgtgttccgggacgccagcagattcatcctgaacctgaccagcgtgaagcccgaggacagcggcatctatttctgcatgatcgtgggcagccccgagctgacatttggcaagggaacacagctgtccgtggtggacttcctgcctactacagcccagcctaccaagaagtctaccctgaagaaaagagtgtgcagactgcccagacctgagacacagaaaggccctctgtgcagccctatcacactgggattgctggtggctggcgtgctggtgctgctggtttctctgggagttgccatccacctgtgctgcagaagaagaagggccagactgcggttcatgaagcagcctcaaggcgagggcatcagcggcacatttgtgcctcaatgcctgcacggctactactccaacaccaccaccagccagaagctgctgaacccctggatcctgaaaacaggcagcggcgccaccaacttcagcctgcttaaacaggccggcgacgtggaagagaaccccggacctatggctctgcctgtgacagctctgctgctgcctctggctctgcttctgcatgccgctagacccagccagttcagagtgtcccctctggacagaacctggaacctgggcgagacagtggaactgaagtgccaggtcctgctgagcaatcctaccagcggctgcagctggctgtttcagcctagaggtgctgccgcctctcctacctttctgctgtacctgagccagaacaagcccaaggccgccgaaggactggacacccagagattcagcggcaagagactgggcgacaccttcgtgctgaccctgagcgacttcagaagagagaacgagggctactatttctgtagcgccctgtccaacagcatcatgtacttcagccacttcgtgcccgtgtttctgcccgccaagcctacaacaacccctgctcctagacctcctacaccagctcctacaatcgccagccagcctctgtctctgaggccagaagcctgtagaccagctgctggcggagccgtgcatacaagaggactggatttcgcctgcgacatctacatctgggcccctctggctggaacttgcggagtgctgttgctgagcctggtcatcaccctgtactgcaaccaccggaacaggcggagagtgtgtaaatgccccaggcctgtggtcaagagcggcgataagcctagcctgagcgccagatatgttggctccggcgctacaaatttcagcctcctgaagcaggcaggggatgtcgaagagaatcctggtccaatgggcagcagactgctgtgctgggttctgctgtgtctgcttggagccggacctgtgaaagctggcgtgacccagacacctagatacctgatcaagaccagaggccagcaagtgacactgagctgtagccccatctccggccacagaagcgtgtcctggtatcagcagacaccaggccagggcctgcagttcctgttcgagtacttctccgagactcagcggaacaagggcaacttccccggcagattttccggcagacagttcagcaactcccgcagcgagatgaacgtgtccacactggaactgggagactctgccctgtacctgtgtgcctctagtctcgctggaaccggcgctcacttcatcaccaacgagaagctgttcttcggcagcggcactcagctgtctgtgctggaagatctgcggaacgtgacccctcctaaggtgtccctgtttgagccaagcaaggccgagatcgccaacaagcagaaagccacactcgtgtgcctggccagaggcttctttcccgatcacgtggaactgtcttggtgggtcaacggcaaagaggtgcacagcggcgtctgtactgatcctcaggcctacaaagagagcaactacagctactgcctgtcctccagactgagagtgtccgccaccttctggcacaaccccagaaaccacttcagatgccaggtgcagtttcacggcctgagcgaagaggacaagtggcctgagggaagccccaagccagtgacacagaatatctctgccgaggcatggggcagagccgattgtggaattaccagcgccagctaccatcagggcgtgctgtctgccacaatcctgtacgagatcctgctgggcaaagccactctgtacgcagtgctcgtgtctggactggtgctgatggccatggtcaagaagaaaaacagcggctccggggccactaactttagtctgctgaagcaagctggcgacgttgaagaaaatcctgggcctatgctgctggaacacctcctgatcatcctgtggatgcagctgacatgggtgtccgggcagcagctgaatcagagccctcagagcatgttcatccaagaaggcgaggacgtttccatgaactgcaccagcagctccatcttcaacacctggctgtggtacaagcaagagcctggcgaaggacccgtgctgctgatcgctctttacaaagccggcgagctgaccagcaacggcagactgacagcccagttcggcattacccggaaggacagcttcctgaacatcagcgctagcatccccagcgacgtgggcatctacttttgcgccggacaactgtggggcggctccaattacaagctgacatttggaaagggcaccctgctgaccgtgaatcccaacattcagaaccccgagcctgccgtgtaccagctgaaggatcctagaagccaggacagcaccctgtgcctgttcaccgacttcgacagccagatcaacgtgcccaagaccatggaatccggcacctttatcaccgataagtgcgtgctggacatgaaggccatggacagcaagagcaacggcgccattgcctggtctaaccagaccagcttcacgtgccaggacatcttcaaagagacaaacgccacctatcctagctccgacgtgccctgtgatgccacactgaccgagaagtccttcgagacagacatgaacctgaacttccagaacctgagcgtgatgggcctgcgcatcctgctgctgaaagtggccggcttcaacctgctgatgaccctgcgactgtggtccagc

SEQ ID NO: 15 - DNA, 566 bp, synthetic construct
  source 1..566: mol_type = other DNA; note = IRES
gtggcggctagtactccggtattgcggtacccttgtacgcctgttttatactcccttcccgtaacttagacgcacaaaaccaagttcaatagaagggggtacaaaccagtaccaccacgaacaagcacttctgtttccccggtgatgtcgtatagactgcttgcgtggttgaaagcgacggatccgttatccgcttatgtacttcgagaagcccagtaccacctcggaatcttcgatgcgttgcgctcagcactcaaccccagagtgtagcttaggctgatgagtctggacatccctcaccggtgacggtggtccaggctgcgttggcggcctacctatggctaacgccatgggacgctagttgtgaacaaggtgtgaagagcctattgagctacataagaatcctccggcccctgaatgcggctaatcccaacctcggagcaggtggtcacaaaccagtgattggcctgtcgtaacgcgcaagtccgtggcggaaccgactactttgggtgtccgtgtttccttttattttattgtggctgcttatggtgacaatcacagattgt

SEQ ID NO: 16 - protein, 210 aa, Homo sapiens
  source 1..210: note = amino acid sequence of human CD8 beta chain isoform 1
MRPRLWLLLAAQLTVLHGNSVLQQTPAYIKVQTNKMVMLSCEAKISLSNMRIYWLRQRQAPSSDSHHEFLALWDSAKGTIHGEEVEQEKIAVFRDASRFILNLTSVKPEDSGIYFCMIVGSPELTFGKGTQLSVVDFLPTTAQPTKKSTLKKRVCRLPRPETQKGPLCSPITLGLLVAGVLVLLVSLGVAIHLCCRRRRARLRFMKQFYK

SEQ ID NO: 17 - protein, 221 aa, Homo sapiens
  source 1..221: note = amino acid sequence of human CD8 beta chain isoform 2
MRPRLWLLLAAQLTVLHGNSVLQQTPAYIKVQTNKMVMLSCEAKISLSNMRIYWLRQRQAPSSDSHHEFLALWDSAKGTIHGEEVEQEKIAVFRDASRFILNLTSVKPEDSGIYFCMIVGSPELTFGKGTQLSVVDFLPTTAQPTKKSTLKKRVCRLPRPETQKGPLCSPITLGLLVAGVLVLLVSLGVAIHLCCRRRRARLRFMKQLRLHPLEKCSRMDY

SEQ ID NO: 18 - protein, 213 aa, Homo sapiens
  source 1..213: note = amino acid sequence of human CD8 beta chain isoform 3
MRPRLWLLLAAQLTVLHGNSVLQQTPAYIKVQTNKMVMLSCEAKISLSNMRIYWLRQRQAPSSDSHHEFLALWDSAKGTIHGEEVEQEKIAVFRDASRFILNLTSVKPEDSGIYFCMIVGSPELTFGKGTQLSVVDFLPTTAQPTKKSTLKKRVCRLPRPETQKGRRRRARLRFMKQPQGEGISGTFVPQCLHGYYSNTTTSQKLLNPWILKT

SEQ ID NO: 19 - protein, 246 aa, Homo sapiens
  source 1..246: note = amino acid sequence of human CD8 beta chain isoform 4
MRPRLWLLLAAQLTVLHGNSVLQQTPAYIKVQTNKMVMLSCEAKISLSNMRIYWLRQRQAPSSDSHHEFLALWDSAKGTIHGEEVEQEKIAVFRDASRFILNLTSVKPEDSGIYFCMIVGSPELTFGKGTQLSVVDFLPTTAQPTKKSTLKKRVCRLPRPETQKGPLCSPITLGLLVAGVLVLLVSLGVAIHLCCRRRRARLRFMKQKFNIVCLKISGFTTCCCFQILQISREYGFGVLLQKDIGQ

SEQ ID NO: 20 - protein, 180 aa, Homo sapiens
  source 1..180: note = amino acid sequence of human CD8 beta chain isoform 6
MRPRLWLLLAAQLTVLHGNSVLQQTPAYIKVQTNKMVMLSCEAKISLSNMRIYWLRQRQAPSSDSHHEFLALWDSAKGTIHGEEVEQEKIAVFRDASRFILNLTSVKPEDSGIYFCMIVGSPELTFGKGTQLSVVDFLPTTAQPTKKSTLKKRVCRLPRPETQKGRRRRARLRFMKQFYK

SEQ ID NO: 21 - protein, 206 aa, Homo sapiens
  source 1..206: note = amino acid sequence of human CD8 beta chain isoform 7
MRPRLWLLLAAQLTVLHGNSVLQQTPAYIKVQTNKMVMLSCEAKISLSNMRIYWLRQRQAPSSDSHHEFLALWDSAKGTIHGEEVEQEKIAVFRDASRFILNLTSVKPEDSGIYFCMIVGSPELTFGKGTQLSVVDFLPTTAQPTKKSTLKKRVCRLPRPETQKDFTNKQRIGFWCPATKRHRSVMSTMWKNERRDTFNPGEFNGC

SEQ ID NO: 22 - protein, 198 aa, Homo sapiens
  source 1..198: note = amino acid sequence of human CD8 beta chain isoform 8
MRPRLWLLLAAQLTVLHGNSVLQQTPAYIKVQTNKMVMLSCEAKISLSNMRIYWLRQRQAPSSDSHHEFLALWDSAKGTIHGEEVEQEKIAVFRDASRFILNLTSVKPEDSGIYFCMIVGSPELTFGKGTQLSVVDFLPTTAQPTKKSTLKKRVCRLPRPETQKGLKGKVYQEPLSPNACMDTTAILQPHRSCLTHGS

SEQ ID NO: 23 - protein, 198 aa, Homo sapiens
  source 1..198: note = amino acid sequence of human CD8 alpha chain isoform 2
MALPVTALLLPLALLLHAARPSQFRVSPLDRTWNLGETVELKCQVLLSNPTSGCSWLFQPRGAAASPTFLLYLSQNKPKAAEGLDTQRFSGKRLGDTFVLTLSDFRRENEGYYFCSALSNSIMYFSHFVPVFLPAKPTTTPAPRPPTPAPTIASQPLSLRPEACRPAAGGAGNRRRVCKCPRPVVKSGDKPSLSARYV

SEQ ID NO: 24 - protein, 276 aa, Homo sapiens
  source 1..276: note = amino acid sequence of human CD8 alpha chain isoform 3
MRNQAPGRPKGATFPPRRPTGSRAPPLAPELRAKQRPGERVMALPVTALLLPLALLLHAARPSQFRVSPLDRTWNLGETVELKCQVLLSNPTSGCSWLFQPRGAAASPTFLLYLSQNKPKAAEGLDTQRFSGKRLGDTFVLTLSDFRRENEGYYFCSALSNSIMYFSHFVPVFLPAKPTTTPAPRPPTPAPTIASQPLSLRPEACRPAAGGAVHTRGLDFACDIYIWAPLAGTCGVLLLSLVITLYCNHRNRRRVCKCPRPVVKSGDKPSLSARYV